European Patent Application EP 4 512 824 A1, published February 26, 2025. Title: BIOSYNTHESIS-BASED PREPARATION METHOD FOR STRUCTURAL MATERIAL OF HUMAN BODY. Applicant: SHANXI JINBO BIO-PHARMACEUTICAL CO., LTD. Application EP, filed April 10, 2023. The sequence listing filed with the application follows.

SEQUENCE LISTING (22 sequences)

SEQ ID NO: 1 - protein, 36 aa, Homo sapiens
GKEGTKGDPGPAGLPGKDGPPGLRGFPGDRGLPGPV

SEQ ID NO: 2 - protein, 39 aa, Homo sapiens
GKEGTKGDPGPAGLPGKDGPPGLRGFPGDRGLPGPVGAL

SEQ ID NO: 3 - protein, 42 aa, Homo sapiens
GKEGTKGDPGPAGLPGKDGPPGLRGFPGDRGLPGPVGALGLK

SEQ ID NO: 4 - protein, 360 aa, synthetic construct
GKEGTKGDPGPAGLPGKDGPPGLRGFPGDRGLPGPVGKEGTKGDPGPAGLPGKDGPPGLRGFPGDRGLPGPVGKEGTKGDPGPAGLPGKDGPPGLRGFPGDRGLPGPVGKEGTKGDPGPAGLPGKDGPPGLRGFPGDRGLPGPVGKEGTKGDPGPAGLPGKDGPPGLRGFPGDRGLPGPVGKEGTKGDPGPAGLPGKDGPPGLRGFPGDRGLPGPVGKEGTKGDPGPAGLPGKDGPPGLRGFPGDRGLPGPVGKEGTKGDPGPAGLPGKDGPPGLRGFPGDRGLPGPVGKEGTKGDPGPAGLPGKDGPPGLRGFPGDRGLPGPVGKEGTKGDPGPAGLPGKDGPPGLRGFPGDRGLPGPV

SEQ ID NO: 5 - protein, 312 aa, synthetic construct
GKEGTKGDPGPAGLPGKDGPPGLRGFPGDRGLPGPVGALGKEGTKGDPGPAGLPGKDGPPGLRGFPGDRGLPGPVGALGKEGTKGDPGPAGLPGKDGPPGLRGFPGDRGLPGPVGALGKEGTKGDPGPAGLPGKDGPPGLRGFPGDRGLPGPVGALGKEGTKGDPGPAGLPGKDGPPGLRGFPGDRGLPGPVGALGKEGTKGDPGPAGLPGKDGPPGLRGFPGDRGLPGPVGALGKEGTKGDPGPAGLPGKDGPPGLRGFPGDRGLPGPVGALGKEGTKGDPGPAGLPGKDGPPGLRGFPGDRGLPGPVGAL

SEQ ID NO: 6 - protein, 336 aa, synthetic construct
GKEGTKGDPGPAGLPGKDGPPGLRGFPGDRGLPGPVGALGLKGKEGTKGDPGPAGLPGKDGPPGLRGFPGDRGLPGPVGALGLKGKEGTKGDPGPAGLPGKDGPPGLRGFPGDRGLPGPVGALGLKGKEGTKGDPGPAGLPGKDGPPGLRGFPGDRGLPGPVGALGLKGKEGTKGDPGPAGLPGKDGPPGLRGFPGDRGLPGPVGALGLKGKEGTKGDPGPAGLPGKDGPPGLRGFPGDRGLPGPVGALGLKGKEGTKGDPGPAGLPGKDGPPGLRGFPGDRGLPGPVGALGLKGKEGTKGDPGPAGLPGKDGPPGLRGFPGDRGLPGPVGALGLK

SEQ ID NO: 7 - protein, 6 aa, Homo sapiens
GALGLK

SEQ ID NO: 8 - protein, 37 aa, Homo sapiens
GKEGTKGDPGPAGLPGKDGPPGLRGFPGDRGLPGPVG

SEQ ID NO: 9 - protein, 38 aa, Homo sapiens
GKEGTKGDPGPAGLPGKDGPPGLRGFPGDRGLPGPVGA

SEQ ID NO: 10 - protein, 40 aa, Homo sapiens
GKEGTKGDPGPAGLPGKDGPPGLRGFPGDRGLPGPVGALG

SEQ ID NO: 11 - protein, 41 aa, Homo sapiens
GKEGTKGDPGPAGLPGKDGPPGLRGFPGDRGLPGPVGALGL

SEQ ID NO: 12 - DNA, 1011 bp, synthetic construct
  source 1..1011: mol_type = other DNA
gggaaagaaggaacgaaaggtgaccctggcccagcgggtctgccgggcaaggacggtccaccgggtctgcgcggtttcccgggcgaccgcggcctgccgggtccggttggcgcgttgggtcttaagggcaaagaaggcaccaaaggagatccgggtccggctggtttaccgggcaaggatggtccgccgggtctgcgtggttttccgggtgaccgtggtctgccgggtccggtcggagccctgggtttgaagggcaaagagggcaccaaaggcgacccaggaccggcaggcctcccgggtaaggatggccctccggggctgcgtggttttccgggtgatcgcggcttgccgggaccggttggtgcgctgggtcttaagggtaaagaaggcaccaaaggtgacccgggcccggcgggtctgccgggcaaagatggtccgccaggcctgagaggcttcccgggtgaccgcggcttgccgggtccggttggtgcgctgggccttaagggtaaagagggcaccaaaggcgatccgggtccggctggcctgccggggaaggacggcccaccgggcctgcgtggttttccgggcgaccgtggtttgccgggcccggtgggcgctctgggtctgaaagggaaagagggtacgaagggtgatccgggtccggcaggcttgccgggcaaggacggcccgcctggcctgcgtggtttcccgggtgaccgtggtttaccgggtcccgtgggcgcgctgggtctgaaaggtaaggaaggcaccaagggtgatccgggcccggccggtctgccgggcaaggacggtccgcccggattacgtggcttcccgggtgatcgtggtctgccgggtcctgtaggtgcgctgggtctcaagggcaaagagggtactaagggtgatccgggcccggcgggtctgccaggcaaagacggcccaccgggcttgcgcggttttccgggcgatcgtggtttgccgggtcctgtgggcgcactgggcttgaagtaa

SEQ ID NO: 13 - DNA, 939 bp, synthetic construct
  source 1..939: mol_type = other DNA
gggaaagaaggaaccaagggtgacccggggccagccggtttgccgggtaaggatggtccgcctggcttgcgtggttttccgggggaccgtggtttgccgggtccggttggtgcgctgggtaaagaaggcacgaagggcgacccgggcccagccggtttaccggggaaagatggtcctccgggcctgcgcggttttccgggagaccgtggtcttccgggcccggtgggtgcgctgggcaaggagggcaccaaaggtgaccctggccctgcgggtctgccgggtaaggacggtccaccgggtctgcgtggctttccgggcgaccgtggcttgcccggtccggttggcgcgctgggtaaagagggtacgaagggtgacccgggtcctgcgggcctgccgggcaaggacggcccgccgggactgcgcggattcccgggcgatcgcggcctcccgggtccggtcggtgcgctgggcaaagaaggtactaaaggtgatccgggcccggcgggcctgccgggcaaggatggcccgccgggtttgcgcggtttcccgggcgaccgtggtttgccgggcccagtgggcgcactgggtaaggagggcaccaaaggcgatccgggaccagctggtctgccgggcaaggacggcccaccgggtctcagaggcttcccgggggaccgcggtctgccgggcccggtaggcgcactgggtaaagaaggcaccaaaggtgacccgggtccggctggtctgccgggtaaggatggcccgccgggcctgcgtggcttcccgggtgatcgtggcttgcctggcccagtgggtgcactgggcaaagagggcaccaagggtgatccgggtccggcgggtctgccgggtaaagatggtccaccgggtttacgtggttttccgggcgatcgtggtctcccgggcccggttggcgctctgtaa

SEQ ID NO: 14 - DNA, 1083 bp, synthetic construct
  source 1..1083: mol_type = other DNA
gggaaagaaggaacgaaaggcgatccgggtccggcgggcctgccgggtaaggacggcccgccgggattacgcggtttcccgggtgaccgcggtttgccgggtccggttggcaaagaaggtactaagggtgatccgggcccagccggtctgccgggcaaggatggtccgccaggcctgagaggcttcccgggtgaccgcgggctgccgggcccggttggtaaggagggcaccaaaggcgatccgggtccggcgggtttgccgggcaaggatggcccgccaggcctgcgtggctttccgggtgatcgtggtctgccgggccccgtgggcaaagagggcaccaaaggtgatccgggtccagcgggtctgccaggtaaggacggtccgcctggcctgcgtggtttcccgggtgatcgtggtctgccgggtccggtcggtaaagaaggcaccaagggcgacccgggcccggcagggctgccgggtaaggatggcccaccgggtctgcgtggttttccgggcgaccgtggtcttccgggtccggtcggtaaagagggcaccaaaggtgacccgggtcccgcgggtctgccgggtaaggacggccctccgggcctgcgcggcttcccgggcgatcgcggtctgccgggtccggttggtaaagaaggtacgaagggcgatcctggtccagcaggcttgccgggcaaagatggtccgcccggccttcgcggattcccgggcgaccgtggcctgccgggtccggtgggtaaagaaggcaccaagggcgacccgggtcctgctggcttgccgggcaaggacggcccaccgggtttacgcggttttccgggcgatcgtggtttgccgggtccggtgggcaaagagggaaccaaaggtgaccctggcccagctggcttgccgggcaaagatggtccgccgggtctgcgtggctttccgggtgaccgtggtttgccgggcccggttggtaaggagggcaccaaaggcgacccgggtccggcgggtctgccgggtaaggacggtccaccgggcttacgtggtttcccgggggaccgtggcctgccgggccccgtgtaa

SEQ ID NO: 15 - protein, 17 aa, synthetic construct
GKEGTKGDPGPAGLPGK

SEQ ID NO: 16 - protein, 22 aa, synthetic construct
EGTKGDPGPAGLPGKDGPPGLR

SEQ ID NO: 17 - protein, 18 aa, synthetic construct
GDPGPAGLPGKDGPPGLR

SEQ ID NO: 18 - protein, 7 aa, synthetic construct
DGPPGLR

SEQ ID NO: 19 - protein, 18 aa, synthetic construct
GFPGDRGLPGPVGALGLK

SEQ ID NO: 20 - protein, 12 aa, synthetic construct
GLPGPVGALGLK

SEQ ID NO: 21 - protein, 11 aa, synthetic construct
GLPGPVGALGK

SEQ ID NO: 22 - protein, 14 aa, synthetic construct
GFPGDRGLPGPVGK